European Patent Specification EP 4 038 205 B1, published July 3, 2024. Title: Clinical and Molecular Prognostic Markers for Liver Transplantation. Applicant: Ophiomics. The sequence listing filed with the application follows.

SEQUENCE LISTING (34 sequences)

SEQ ID NO: 1 - DNA, 19 bp, Artificial Sequence
  Primer
ctggaagcaccggaaggag

SEQ ID NO: 2 - DNA, 22 bp, Artificial Sequence
  Primer
ccatatgttctccagagcgcag

SEQ ID NO: 3 - DNA, 24 bp, Artificial Sequence
  Primer
attccaggtctatggaaatgcagg

SEQ ID NO: 4 - DNA, 23 bp, Artificial Sequence
  Primer
cgtcagatccccaaaaagaaaat

SEQ ID NO: 5 - DNA, 18 bp, Artificial Sequence
  Primer
gcaacaacgacgccgaat

SEQ ID NO: 6 - DNA, 18 bp, Artificial Sequence
  Primer
ccgcgatcacggagttca

SEQ ID NO: 7 - DNA, 17 bp, Artificial Sequence
  Primer
aactacgcctgcatgcc

SEQ ID NO: 8 - DNA, 17 bp, Artificial Sequence
  Primer
ctacgtgccctgcagcc

SEQ ID NO: 9 - DNA, 18 bp, Artificial Sequence
  Primer
gcctgtgagctgaagggg

SEQ ID NO: 10 - DNA, 20 bp, Artificial Sequence
  Primer
actctgctgctgtttgtggg

SEQ ID NO: 11 - DNA, 23 bp, Artificial Sequence
  Primer
gactcacacactggagagaagcc

SEQ ID NO: 12 - DNA, 20 bp, Artificial Sequence
  Primer
gttgtgacacgacaccctga

SEQ ID NO: 13 - DNA, 20 bp, Artificial Sequence
  Primer
gggacatgggcagagcaatg

SEQ ID NO: 14 - DNA, 18 bp, Artificial Sequence
  Primer
cacccaggctctgcagtc

SEQ ID NO: 15 - DNA, 21 bp, Artificial Sequence
  Primer
gatgctcagtgaggacccttg

SEQ ID NO: 16 - DNA, 21 bp, Artificial Sequence
  Primer
cctacctttcacctggtagcc

SEQ ID NO: 17 - DNA, 19 bp, Artificial Sequence
  Primer
ccttcgatggagtgccagg

SEQ ID NO: 18 - DNA, 23 bp, Artificial Sequence
  Primer
gtaaatgtccgatttcgtgagcc

SEQ ID NO: 19 - DNA, 23 bp, Artificial Sequence
  Primer
cagtttggagctacctggagtat

SEQ ID NO: 20 - DNA, 22 bp, Artificial Sequence
  Primer
aagtagcccacaagagtaagca

SEQ ID NO: 21 - DNA, 20 bp, Artificial Sequence
  Primer
gtccactccagctctgaaac

SEQ ID NO: 22 - DNA, 19 bp, Artificial Sequence
  Primer
ccactctgagctctggcct

SEQ ID NO: 23 - DNA, 20 bp, Artificial Sequence
  Primer
gcacgtctggtaccattcca

SEQ ID NO: 24 - DNA, 16 bp, Artificial Sequence
  Primer
ccggtgaagcctggca

SEQ ID NO: 25 - DNA, 23 bp, Artificial Sequence
  Primer
cattgattccccgcttcattgtg

SEQ ID NO: 26 - DNA, 22 bp, Artificial Sequence
  Primer
tggacatttcctggagctcatt

SEQ ID NO: 27 - DNA, 23 bp, Artificial Sequence
  Primer
catgtagtgaacctttaagttgc

SEQ ID NO: 28 - DNA, 17 bp, Artificial Sequence
  Primer
atccatcacggccacca

SEQ ID NO: 29 - DNA, 22 bp, Artificial Sequence
  Primer
ataaatctgcgtgggtaggagc

SEQ ID NO: 30 - DNA, 20 bp, Artificial Sequence
  Primer
gggtacggctggtagttgtc

SEQ ID NO: 31 - DNA, 19 bp, Artificial Sequence
  Primer
ggtgacatcgaccacctcc

SEQ ID NO: 32 - DNA, 24 bp, Artificial Sequence
  Primer
gtctcaaggatacctgctacagaa

SEQ ID NO: 33 - DNA, 20 bp, Artificial Sequence
  Primer
cgtgcgaggtatgctgcccc

SEQ ID NO: 34 - DNA, 20 bp, Artificial Sequence
  Primer
ggcggtgggatgccgtcaaa